European Patent Application EP 4 559 931 A1, published May 28, 2025. Title: ANTI-RESPIRATORY SYNCYTIAL VIRUS NEUTRALIZING ANTIBODY AND USE THEREOF. Applicant: Beijing Wisdomab Biotechnology Co., Ltd. Application EP 23841910.5, filed May 30, 2023. The sequence listing filed with the application follows.

SEQUENCE LISTING (46 sequences)

SEQ ID NO: 1 - DNA, 190 bp, Escherichia coli
  source 1..190: mol_type = genomic DNA
cgaataaatacctgtgacggaagatcacttcgcagaataaataaatcctggtgtccctgttgataccgggaagccctgggccaacttttggcgaaaatgagacgttgatcggcacgtaagaggttccaactttcaccataatgaaataagatcactaccgggcgtattttttgagttatcgagattttca

SEQ ID NO: 2 - DNA, 232 bp, Lambda phage targeting Escherichia
  source 1..232: mol_type = genomic DNA
aaataatgattttattttgactgatagtgacctgttcgttgcaacacattgatgagcaatgcttttttataatgccaactttgtacaaaaaagctgaacgagaaacgtaaaatgatataaatatcaatatattaaattagattttgcataaaaaacagactacataatactgtaaaacacaacatatccagtcactatgaatcaactacttagatggtattagtgacctgta

SEQ ID NO: 3 - DNA, 739 bp, Escherichia coli
  source 1..739: mol_type = genomic DNA
gatcaaaggatcttcttgagatcctttttttctgcgcgtaatcttttgccctgtaaacgaaaaaaccacctggggaggtggtttgatcgaaggttaagtcagttggggaactgcttaaccgtggtaactggttttcgcagagcacagcaaccaaatctgtccttccagtgtagccggactttggcgcacacttcaagagcaaccgcgtgtttagctaaacaaatcctctgcgaactcccagttaccaatggctgctgccagtggcgttttaccgtgcttttccgggttggactcaagtgaacagttaccggataaggcgcagcagtcgggctgaacggggagttcttgcttacagcccagcttggagcgaacgacctacaccgagccgagataccagtgtgtgagctatgagaaagcgccacacttcccgtaagggagaaaggcggaacaggtatccggtaaacggcagggtcggaacaggagagcgcaagagggagcgacccgccggaaacggtggggatctttaagtcctgtcgggtttcgcccgtactgtcagattcatggttgagcctcacggctcccacagatgcaccggaaaagcgtctgtttatgtgaactctggcaggagggcggagcctatggaaaaacgccaccggcgcggccctgctgttttgcctcacatgttagtcccctgcttatccacggaatctgtgggtaactttgtatgtgtccgcagcgc

SEQ ID NO: 4 - DNA, 25 bp, Escherichia coli
  source 1..25: mol_type = genomic DNA
acaagtttgtacaaaaaagcaggct

SEQ ID NO: 5 - DNA, 660 bp, Escherichia coli
  source 1..660: mol_type = genomic DNA
atggagaaaaaaatcactggatataccaccgttgatatatcccaatggcatcgtaaagaacattttgaggcatttcagtcagttgctcaatgtacctataaccagaccgttcagctggatattacggcctttttaaagaccgtaaagaaaaataagcacaagttttatccggcctttattcacattcttgcccgcctgatgaatgctcatccggaattccgtatggcaatgaaagacggtgagctggtgatatgggatagtgttcacccttgttacaccgttttccatgagcaaactgaaacgttttcatcgctctggagtgaataccacgacgatttccggcagtttctacacatatattcgcaagatgtggcgtgttacggtgaaaacctggcctatttccctaaagggtttattgagaatatgtttttcgtctcagccaatccctgggtgagtttcaccagttttgatttaaacgtggccaatatggacaacttcttcgcccccgttttcactatgggcaaatattatacgcaaggcgacaaggtgctgatgccgctggcgattcaggttcatcatgccgtctttgatggcttccatgtcggcagaatgcttaatgaattacaacagtactgcgatgagtggcagggcggggcgtaa

SEQ ID NO: 6 - DNA, 1163 bp, Escherichia coli
  source 1..1163: mol_type = genomic DNA
tcaggtggcacttttcggggaaatgtgcgcggaacccctatttgtttatttttctaaatacattcaaatatgtatccgctcatgagacaataaccctgataaatgcttcaataatattgaaaaaggaagagtatgagtattcaacatttccgtgtcgcccttattcccttttttgcggcattttgccttcctgtttttgctcacccagaaacgctggtgaaagtaaaagatgctgaagatcagttgggtgcacgagtgggttacatcgaactggatctcaacagcggtaagatccttgagagttttcgccccgaagaacgttttccaatgatgagcacttttaaagttctgctatgtggcgcggtattatcccgtattgacgccgggcaagagcaactcggtcgccgcatacactattctcagaatgacttggttgagtactcaccagtcacagaaaagcatcttacggatggcatgacagtaagagaattatgcagtgctgccataaccatgagtgataacactgcggccaacttacttctgacaacgatcggaggaccgaaggagctaaccgcttttttgcacaacatgggggatcatgtaactcgccttgatcgttgggaaccggagctgaatgaagccataccaaacgacgagcgtgacaccacgatgcctgtagcaatggcaacaacgttgcgcaaactattaactggcgaactacttactctagcttcccggcaacaattaatagactggatggaggcggataaagttgcaggaccacttctgcgctcggcccttccggctggctggtttattgctgataaatctggagccggtgagcgtgggtctcgcggtatcattgcagcactggggccagatggtaagccctcccgtatcgtagttatctacacgacggggagtcaggcaactatggatgaacgaaatagacagatcgctgagataggtgcctcactgattaagcattggtaactgtcagaccaagtttactcatatatactttagattgatttaaaacttcatttttaatttaaaaggatctaggtgaagatcctttttgataatctcatgaccaaaatcccttaacgtgagttttcgttccactgagcgtcagaccccgtagaaaagatcaaaggatcttc

SEQ ID NO: 7 - DNA, 1760 bp, Lambda phage targeting Escherichia
  source 1..1760: mol_type = genomic DNA
ctggcacgacaggtttcccgactggaaagcgggcagtgagcgcaacgcaattaatgtaagttagctcactcattaggcaccccaggctttacactttatgcttccggctcgtataatgtgtggaattgtgagcggataacaatttcacacaggaaacagctatgaccatgattacggattcactggccgtcgttttacaacgtcgtgactgggaaaaccctggcgttacccaacttaatcgccttgcagcacatccccctttcgccagctggcgtaatagcgaagaggcccgcaccgatcgcccttcccaacagttgcgcagcctgaatggcgaatggcgctttgcctggtttccggcaccagaagcggtgccggaaagctggctggagtgcgatcttcctgaggccgatactgtcgtcgtcccctcaaactggcagatgcacggttacgatgcgcccatctacaccaacgtgacctatcccattacggtcaatccgccgtttgttcccacggagaatccgacgggttgttactcgctcacatttaatgttgatgaaagctggctacaggaaggccagacgcgaattatttttgatggcgtcgggatctgatccggatttactaactggaagaggcactaaatgggaagaaggcgaagtcatgagcgccgggatttaccccctaacctttatataagaaacaatggatattactgctacagggacccaaggacgggtaaagagtttggattaggcagagacaggcgaatcgcaatcactgaagctatacaggccaacattgagttattttcaggacacaaacacaagcctctgacagcgagaatcaacagtgataattccgttacgttacattcatggcttgatcgctacgaaaaaatcctggccagcagaggaatcaagcagaagacactcataaattacatgagcaaaattaaagcaataaggaggggtctgcctgatgctccacttgaagacatcaccacaaaagaaattgcggcaatgctcaatggatacatagacgagggcaaggcggcgtcagccaagttaatcagatcaacactgagcgatgcattccgagaggcaatagctgaaggccatataacaacaaaccatgtcgctgccactcgcgcagcaaaatcagaggtaaggagatcaagacttacggctgacgaatacctgaaaatttatcaagcagcagaatcatcaccatgttggctcagacttgcaatggaactggctgttgttaccgggcaacgagttggtgatttatgcgaaatgaagtggtctgatatcgtagatggatatctttatgtcgagcaaagcaaaacaggcgtaaaaattgccatcccaacagcattgcatattgatgctctcggaatatcaatgaaggaaacacttgataaatgcaaagagattcttggcggagaaaccataattgcatctactcgtcgcgaaccgctttcatccggcacagtatcaaggtattttatgcgcgcacgaaaagcatcaggtctttccttcgaaggggatccgcctacctttcacgagttgcgcagtttgtctgcaagactctatgagaagcagataagcgataagtttgctcaacatcttctcgggcataagtcggacaccatggcatcacagtatcgtgatgacagaggcagggagtgggacaaaattgaaatcaaataactagcataaccccttggggcctctaaacgggtcttgaggggttttttg

SEQ ID NO: 8 - DNA, 99 bp, synthetic construct
  source 1..99: mol_type = other DNA
aaataatgattttattttgactgatagtgacctgttcgttgcaacacattgatgagcaatgcttttttataatgccaactttgtacaaaaaagcaggct

SEQ ID NO: 9 - DNA, 158 bp, synthetic construct
  source 1..158: mol_type = other DNA
acaagtttgtacaaaaaagctgaacgagaaacgtaaaatgatataaatatcaatatattaaattagattttgcataaaaaacagactacataatactgtaaaacacaacatatccagtcactatgaatcaactacttagatggtattagtgacctgta

SEQ ID NO: 10 - protein, 574 aa, strain A2 of subtype A RSV
MELLILKANAITTILTAVTFCFASGQNITEEFYQSTCSAVSKGYLSALRTGWYTSVITIELSNIKENKCNGTDAKVKLIKQELDKYKNAVTELQLLMQSTPPTNNRARRELPRFMNYTLNNAKKTNVTLSKKRKRRFLGFLLGVGSAIASGVAVSKVLHLEGEVNKIKSALLSTNKAVVSLSNGVSVLTSKVLDLKNYIDKQLLPIVNKQSCSISNIETVIEFQQKNNRLLEITREFSVNAGVTTPVSTYMLTNSELLSLINDMPITNDQKKLMSNNVQIVRQQSYSIMSIIKEEVLAYVVQLPLYGVIDTPCWKLHTSPLCTTNTKEGSNICLTRTDRGWYCDNAGSVSFFPQAETCKVQSNRVFCDTMNSLTLPSEINLCNVDIFNPKYDCKIMTSKTDVSSSVITSLGAIVSCYGKTKCTASNKNRGIIKTFSNGCDYVSNKGMDTVSVGNTLYYVNKQEGKSLYVKGEPIINFYDPLVFPSDEFDASISQVNEKINQSLAFIRKSDELLHNVNAGKSTTNIMITTIIIVIIVILLSLIAVGLLLYCKARSTPVTLSKDQLSGINNIAFSN

SEQ ID NO: 11 - protein, 574 aa, strain 18537 of subtype B RSV
MELLIHRSSAIFLTLAVNALYLTSSQNITEEFYQSTCSAVSRGYFSALRTGWYTSVITIELSNIKETKCNGTDTKVKLIKQELDKYKNAVTELQLLMQNTPAANNRARREAPQYMNYTINTTKNLNVSISKKRKRRFLGFLLGVGSAIASGIAVSKVLHLEGEVNKIKNALLSTNKAVVSLSNGVSVLTSKVLDLKNYINNRLLPIVNQQSCRISNIETVIEFQQMNSRLLEITREFSVNAGVTTPLSTYMLTNSELLSLINDMPITNDQKKLMSSNVQIVRQQSYSIMSIIKEEVLAYVVQLPIYGVIDTPCWKLHTSPLCTTNIKEGSNICLTRTDRGWYCDNAGSVSFFPQADTCKVQSNRVFCDTMNSLTLPSEVSLCNTDIFNSKYDCKIMTSKTDISSSVITSLGAIVSCYGKTKCTASNKNRGIIKTFSNGCDYVSNKGVDTVSVGNTLYYVNKLEGKNLYVKGEPIINYYDPLVFPSDEFDASISQVNEKINQSLAFIRRSDELLHNVNTGKSTTNIMITTIIIVIIVVLLSLIAIGLLLYCKAKNTPVTLSKDQLSGINNIAFSK

SEQ ID NO: 12 - protein, 544 aa, synthetic construct
MELLILKANAITTILTAVTFCFASGQNITEEFYQSTCSAVSKGYLSALRTGWYTSVITIELSNIKENKCNGTDAKVKLIKQELDKYKNAVTELQLLMQSTPPTNNRARRELPRFMNYTLNNAKKTNVTLSKKRKRRFLGFLLGVGSAIASGVAVCKVLHLEGEVNKIKSALLSTNKAVVSLSNGVSVLTFKVLDLKNYIDKQLLPILNKQSCSISNIETVIEFQQKNNRLLEITREFSVNAGVTTPVSTYMLTNSELLSLINDMPITNDQKKLMSNNVQIVRQQSYSIMCIIKEEVLAYVVQLPLYGVIDTPCWKLHTSPLCTTNTKEGSNICLTRTDRGWYCDNAGSVSFFPQAETCKVQSNRVFCDTMNSLTLPSEINLCNVDIFNPKYDCKIMTSKTDVSSSVITSLGAIVSCYGKTKCTASNKNRGIIKTFSNGCDYVSNKGMDTVSVGNTLYYVNKQEGKSLYVKGEPIINFYDPLVFPSDEFDASISQVNEKINQSLAFIRKSDELLSAIGGYIPEAPRDGQAYVRKDGEWVLLSTFL

SEQ ID NO: 13 - protein, 544 aa, synthetic construct
MELLIHRSSAIFLTLAVNALYLTSSQNITEEFYQSTCSAVSRGYFSALRTGWYTSVITIELSNIKETKCNGTDTKVKLIKQELDKYKNAVTELQLLMQNTPAANNRARREAPQYMNYTINTTKNLNVSISKKRKRRFLGFLLGVGSAIASGIAVCKVLHLEGEVNKIKNALLSTNKAVVSLSNGVSVLTFKVLDLKNYINNRLLPILNQQSCRISNIETVIEFQQMNSRLLEITREFSVNAGVTTPLSTYMLTNSELLSLINDMPITNDQKKLMSSNVQIVRQQSYSIMCIIKEEVLAYVVQLPIYGVIDTPCWKLHTSPLCTTNIKEGSNICLTRTDRGWYCDNAGSVSFFPQADTCKVQSNRVFCDTMNSLTLPSEVSLCNTDIFNSKYDCKIMTSKTDISSSVITSLGAIVSCYGKTKCTASNKNRGIIKTFSNGCDYVSNKGVDTVSVGNTLYYVNKLEGKNLYVKGEPIINYYDPLVFPSDEFDASISQVNEKINQSLAFIRRSDELLSAIGGYIPEAPRDGQAYVRKDGEWVLLSTFL

SEQ ID NO: 14 - protein, 6 aa, synthetic construct
HHHHHH

SEQ ID NO: 15 - protein, 330 aa, Homo sapiens
ASTKGPSVFPLAPSSKSTSGGTAALGCLVKDYFPEPVTVSWNSGALTSGVHTFPAVLQSSGLYSLSSVVTVPSSSLGTQTYICNVNHKPSNTKVDKRVEPKSCDKTHTCPPCPAPELLGGPSVFLFPPKPKDTLMISRTPEVTCVVVDVSHEDPEVKFNWYVDGVEVHNAKTKPREEQYNSTYRVVSVLTVLHQDWLNGKEYKCKVSNKALPAPIEKTISKAKGQPREPQVYTLPPSREEMTKNQVSLTCLVKGFYPSDIAVEWESNGQPENNYKTTPPVLDSDGSFFLYSKLTVDKSRWQQGNVFSCSVMHEALHNHYTQKSLSLSPGK

SEQ ID NO: 16 - protein, 330 aa, Homo sapiens
ASTKGPSVFPLAPSSKSTSGGTAALGCLVKDYFPEPVTVSWNSGALTSGVHTFPAVLQSSGLYSLSSVVTVPSSSLGTQTYICNVNHKPSNTKVDKRVEPKSCDKTHTCPPCPAPELLGGPSVFLFPPKPKDTLYITREPEVTCVVVDVSHEDPEVKFNWYVDGVEVHNAKTKPREEQYNSTYRVVSVLTVLHQDWLNGKEYKCKVSNKALPAPIEKTISKAKGQPREPQVYTLPPSREEMTKNQVSLTCLVKGFYPSDIAVEWESNGQPENNYKTTPPVLDSDGSFFLYSKLTVDKSRWQQGNVFSCSVMHEALHNHYTQKSLSLSPGK

SEQ ID NO: 17 - protein, 330 aa, Mus musculus
AKTTAPSVYPLAPVCGDTTGSSVTLGCLVKGYFPEPVTLTWNSGSLSSGVHTFPAVLQSDLYTLSSSVTVTSSTWPSQSITCNVAHPASSTKVDKKIEPRGPTIKPCPPCKCPAPNLLGGPSVFIFPPKIKDVLMISLSPIVTCVVVDVSEDDPDVQISWFVNNVEVHTAQTQTHREDYNSTLRVVSALPIQHQDWMSGKEFKCKVNNKDLPAPIERTISKPKGSVRAPQVYVLPPPEEEMTKKQVTLTCMVTDFMPEDIYVEWTNNGKTELNYKNTEPVLDSDGSYFMYSKLRVEKKNWVERNSYSCSVVHEGLHNHHTTKSFSRTPGK

SEQ ID NO: 18 - protein, 107 aa, Homo sapiens [sequence omitted]

SEQ ID NO: 19 - protein, 106 aa, Homo sapiens
GQPKAAPSVTLFPPSSEELQANKATLVCLISDFYPGAVTVAWKADSSPVKAGVETTTPSKQSNNKYAASSYLSLTPEQWKSHRSYSCQVTHEGSTVEKTVAPTECS

SEQ ID NO: 20 - protein, 107 aa, Mus musculus
RADAAPTVSIFPPSSEQLTSGGASVVCFLNNFYPKDINVKWKIDGSERQNGVLNSWTDQDSKDSTYSMSSTLTLTKDEYERHNSYTCEATHKTSTSPIVKSFNRNEC

SEQ ID NO: 21 - protein, 106 aa, Mus musculus
GQPKSSPSVTLFPPSSEELETNKATLVCTITDFYPGVVTVDWKVDGTPVTQGMETTQPSKQSNNKYMASSYLTLTARAWERHSSYSCQVTHEGHTVEKSLSRADCS

SEQ ID NO: 22 - protein, 120 aa, synthetic construct
QVTLRESGPALVKPTQTLTLTCTFSGFSLSTSGMSVGWIRQPPGKALEWLADIWWDDKKDYNPSLKSRLTISKDTSKNQVVLKVTNMDPADTATYYCARSMITNWYFDVWGAGTTVTVSS

SEQ ID NO: 23 - protein, 106 aa, synthetic construct
DIQMTQSPSTLSASVGDRVTITCKCQLSVGYMHWYQQKPGKAPKLWIYDTSKLASGVPSRFSGSGSGTEFTLTISSLQPDDFATYYCFQGSGYPFTFGGGTKLEIK

SEQ ID NO: 24 - protein, 126 aa, Homo sapiens [sequence omitted]

SEQ ID NO: 25 - protein, 107 aa, Homo sapiens [sequence omitted]

SEQ ID NO: 26 - protein, 127 aa, Homo sapiens
EVQLVESGGGLVRPGRSLRLSCTVSGFSFDDSAMSWVRQAPGKGLEWISFIKSKTYGGTKEYAASVKGRFTISRDDSKNIAYLQMNSLKTEDTAVYYCTRGAPYGGNSDYYYGLDVWGQGTTVTVSS

SEQ ID NO: 27 - protein, 107 aa, Homo sapiens
DIQMTQSPSSLSASVGDRVTITCRTSQDVRGALAWYQQKPGKAPKLLIFDASSLETGVPSRFSGSGSGTVFTLTISSLQPEDFAAYYCQQFLDFPFTFGQGTRLEIK

SEQ ID NO: 28 - protein, 126 aa, synthetic construct
QVQLVQSGAEVKKPGSSVKVSCKASGGLLEDYIINWVRQAPGQGLEWMGGIIPVLGTVHYGPKFQGRVTITADESTSTAYMELSSLRSEDTAVYYCATETAIVVTESYRPHFFDNWGQGTLVTVSS

SEQ ID NO: 29 - protein, 107 aa, synthetic construct
DIQMTQSPSSLSASVGDRVTITCQASQDIVNYLNWYQQKPGKAPKLLIYVASNLETGVPSRFSGSGSGTDFTFTISSLQPEDIATYYCQEFAGLALNFGGGTKVEIK

SEQ ID NO: 30 - protein, 126 aa, synthetic construct
QVQLVQSGAEVKKPGSSVMVSCQASGDPLQNYIINWVRQAPGQGPEWMGAIIPALGSAHYGPKFQGRVTITADESTDTAYMELSSLRSEDTAMYYCATETAVIISESYLPHFFDNWGQGTLVTVSS

SEQ ID NO: 31 - protein, 107 aa, synthetic construct
DIQMTQSPSSLSAAVGDRVTITCQASQDIVNYLNWYQQKPGKAPKLLIYVASNLETGVPSRFSGSGSGTDFSLTISSLQPEDVATYYCQEYDSLALAFGGGTKVEIK

SEQ ID NO: 32 - protein, 5 aa, synthetic construct
DYIIN

SEQ ID NO: 33 - protein, 17 aa, synthetic construct
GIIPVLGTVHYGPKFQG

SEQ ID NO: 34 - protein, 17 aa, synthetic construct
ETAIVVTESYRPHFFDN

SEQ ID NO: 35 - protein, 11 aa, synthetic construct
QASQDIVNYLN

SEQ ID NO: 36 - protein, 7 aa, synthetic construct
VASNLET

SEQ ID NO: 37 - protein, 9 aa, synthetic construct
QEFAGLALN

SEQ ID NO: 38 - protein, 5 aa, synthetic construct
NYIIN

SEQ ID NO: 39 - protein, 17 aa, synthetic construct
AIIPALGSAHYGPKFQG

SEQ ID NO: 40 - protein, 17 aa, synthetic construct
ETAVIISESYLPHFFDN

SEQ ID NO: 41 - protein, 11 aa, synthetic construct
QASQDIVNYLN

SEQ ID NO: 42 - protein, 7 aa, synthetic construct
VASNLET

SEQ ID NO: 43 - protein, 9 aa, synthetic construct
QEYDSLALA

SEQ ID NO: 44 - DNA, 589 bp, Escherichia coli
  source 1..589: mol_type = genomic DNA
ttgagatcctttttttctgcgcgtaatctgctgcttgcaaacaaaaaaaccaccgctaccagcggtggtttgtttgccggatcaagagctaccaactctttttccgaaggtaactggcttcagcagagcgcagataccaaatactgtccttctagtgtagccgtagttaggccaccacttcaagaactctgtagcaccgcctacatacctcgctctgctaatcctgttaccagtggctgctgccagtggcgataagtcgtgtcttaccgggttggactcaagacgatagttaccggataaggcgcagcggtcgggctgaacggggggttcgtgcacacagcccagcttggagcgaacgacctacaccgaactgagatacctacagcgtgagctatgagaaagcgccacgcttcccgaagggagaaaggcggacaggtatccggtaagcggcagggtcggaacaggagagcgcacgagggagcttccagggggaaacgcctggtatctttatagtcctgtcgggtttcgccacctctgacttgagcgtcgatttttgtgatgctcgtcaggggggcggagcctatggaaa

SEQ ID NO: 45 - DNA, 455 bp, f1 phage
  source 1..455: mol_type = genomic DNA
cgcgccctgtagcggcgcattaagcgcggcgggtgtggtggttacgcgcagcgtgaccgctacacttgccagcgccctagcgcccgctcctttcgctttcttcccttcctttctcgccacgttcgccggctttccccgtcaagctctaaatcgggggctccctttagggttccgatttagtgctttacggcacctcgaccccaaaaaacttgattagggtgatggttcacgtagtgggccatcgccctgatagacggtttttcgccctttgacgttggagtccacgttctttaatagtggactcttgttccaaactggaacaacactcaaccctatctcggtctattcttttgatttataagggattttgccgatttcggcctattggttaaaaaatgagctgatttaacaaaaatttaacgcgaattttaacaaaatattaacgcttacaattt

SEQ ID NO: 46 - DNA, 477 bp, M13 phage
  source 1..477: mol_type = genomic DNA
ggtggcggctccggttccggtgattttgattatgaaaaaatggcaaacgctaataagggggctatgaccgaaaatgccgatgaaaacgcgctacagtctgacgctaaaggcaaacttgattctgtcgctactgattacggtgctgctatcgatggtttcattggtgacgtttccggccttgctaatggtaatggtgctactggtgattttgctggctctaattcccaaatggctcaagtcggtgacggtgataattcacctttaatgaataatttccgtcaatatttaccttccctccctcaatcggttgaatgtcgcccttttgtctttggcgctggtaaaccatatgaattttctattgattgtgacaaaataaacttattccgtggtgtctttgcgtttcttttatatgttgccacctttatgtatgtattttctacgtttgctaacatactgcgtaataaggagtcttgataa